European Patent Application EP 4 563 592 A1, published June 4, 2025. Title: CHIMERIC TRANSCRIPTIONAL ACTIVATOR AND USE THEREOF. Applicant: NANJING BESTZYME BIO-ENGINEERING CO., LTD. Application EP 23845678.4, filed July 28, 2023. The sequence listing filed with the application follows.

SEQUENCE LISTING (31 sequences)

SEQ ID NO: 1 - protein, 560 aa, synthetic construct
MEFVARQSMNACPFVRSTSTHHLKKLAANSSLAATASHCPVVGPALQQQRYYSQPSKPAQAQTSDIATGIKKDVSPIRMDSNETAFDYNGMYESDLANKRKDNSYRYFNNINRLAKEFPKAHRQTEDDKVTVWCSNDYLGMGRHPEIIKTMKATMDKYGSGAGGTRNIAGHNHAAINLESELACLNKKEAALVFSSCFIANDAIISLLGQKIKNLVIFSDQSNHASMILGVRNSKAKKHIFKHNNLKDLESQLAQYPKSTPKLIAFESVYSMCGSVAPIEKICDLAKRYGALTFLDEVHAVGMYGPHGQGVAEHLDFDLHLQSGIASPSVVDKRTILDRVDMITGTCGKSFGTVGGYVAGSANLIDWLRSYAPGFIFTTTLPPAIMAGTATSVRIVRADIEARIKQQLNTRYVKDSFENLGIPVIPNPSHIVPVLVGNAADAKKASDMLMNKHRIYVQAINYPTVPVGEERLRITPTPGHGKEICDQLISAVDDVFTELNLPRINKWQSQGGHCGVGDANYVPEPNLWTQDQLSLTNQDLHSNVHNPVIEQIETSSGVRL

SEQ ID NO: 2 - protein, 341 aa, synthetic construct
MVHKAEYLDDHPTQISSILSGGYNHPLLREWQHERQLNKNMFIFPLFVTDRPDEEELIPSLPNIKRFGVNKLIPYVGGLVSKGLRAVILFGVPLKPGVKDEEGTAADDPEGPVIQAIKHLRKNFPDLYIITDVCLCEYTSHGHCGILYEDGTINRELSVRRIAAVAVKYAQAGANSVAPSDMTDGRIRDIKEGLLSAGLAHKTFVMSYAAKFSGNLYGPFRDAAGSCPSQGDRKCYQLPSGGKGLAHRALIRDMNEGTDGIIVKPSTFYLDIVADAYQLCKDYPICCYQVSGEYAMLHAAAEKNIVDLKSIAFEAHQGFLRAGARLIISYFTPEFLEWLSE

SEQ ID NO: 3 - protein, 344 aa, synthetic construct
MNQIEQSGPIDCSSLKLGSRKSALAIIQAEIVRQLILKEYPELETKLVSVSTLGDQVQNKALFTFGGKSLWTKELEMLLLESVGGFDQIDMIVHSLKDMPTHLPDEFELGCIIEREDPRDALVVQDGLSYKSLADLPEGAVVGTSSVRRSAQLLKNFPHLKFKSVRGNLQTRLRKLDDPDSEYCCLLLAAAGLIRTGLQHRISMYLNDDVMYHSVGQGALGVEIRKGDQFMKNICEKIGHRTTTLRCLAERALLRYLEGGCSVPIGVSTIYSEDTKELTMNSLVVSCNGRDSVTESMTEVVTTEEQAEDFGERLAQKLIDQGAKRILDEINFNKIKEIKEEGLH

SEQ ID NO: 4 - protein, 265 aa, synthetic construct
MPKAILLKNKTTPKDPYLENFVSSGYSTDFVPLLDHIHMEKSEIIAFLKTDYFLHKTLAFIITSQRAVEMLNECMQILRRTDPEITQIIYSKPVYTVGPATYRILADAGFVDLRGGDKAGNGSILAQIILNDDIYTGIEDSDKHITFFTGETRRDIIPKCLLSNNFQLYEKIVYKTLPRDDIVTRFKSAVDSIDQSQRSSSWVVFFSPQGTEDIVTYLQHTKDQFNIASIGPTTEKYLLSKNLKPKVVAPKPEPISLLLSIQKVH

SEQ ID NO: 5 - protein, 361 aa, synthetic construct
MSRFPELKNDLILRAARGEKVERPPIWIMRQAGRYLPEYHEVKGGRDFFETCRDAEIASEITIQPITHFDGLIDAAIIFSDILVIPQAMGMEVKMVDKVGPQFPNPLRKPSDLDHLKKDVDVLKELDWAFKAISLTRKKLNGRVPLLGFCGAPWTLLVYMTEGGGTKMFRFAKEWIYKFTKESHQLLQQITDVAVEFLAQQVVAGAQMLQVFESWGGELGPDEFDEFSLPYLRQISSKLPLRLKELGITENVPITVFAKGSWYALEQLCDSGYDVVSLDWLFRPSDAVQIANGRIALQGNLDPGTMYGSKETISKKVDKMIKGFGGGKQNYIINFGHGTHPFMDPEQIRWFLQECHRIGSQ

SEQ ID NO: 6 - protein, 325 aa, synthetic construct
MAIDSDINLSSPNDSIRQRMFELIQRKQLEIVAALEAIEGNDTKFRSDSWERGAEGGGGRSMLIQDGRVFEKAGVNISKVHGVLPPQAVSQMRNDHSKLDLPAGTSLKFFACGLSLVIHPHNPHAPTTHLNYRYFETWDETGKPHTWWFGGGADLTPSYLYPEDAKQFHQAHKDALDKHDVSLYPRFKKWCDEYFLIKHRNETRGIGGIFFDDFDEFDAERSLKLVEDCFNAFLESYPAITRKRMDTPSTDAEKNWQQIRRGRYVEFNLVLDRGTQFGLRTPGSRVESILMSLPRTAGWVYDHHPEPGSREEELLQVLQNPIEWV

SEQ ID NO: 7 - protein, 560 aa, synthetic construct
MLKSLAPNSSIAVLGSGISGLTFSFFLNRLRPDVKIHIFEKSKQVGGWIRSEEHETFHFEKGPRTLRGTNTGTLMLLDLLTKIGANDKVLGLHKDSLANKKYLLSPFSDVHGNNAKLLQVPQDFSSFVKFMFDPLSKDLILGLLKEPWQPKLKYSDESVDHFFNRRFATKLSENIVSAIVHGIYAGDVKKLSVKAIFPRLPEMEQESGSIIRYMIAQYRTKKNVKQKVDPFLADYEKLIGTSLSFKNISLFLKNFPMLSFQGGLQKLPISLKNHLSQIENIKFHFDSKIKNIALESGKVALTDHDQVYLVDHVRSTINTNELAKIISPVVPSSTKKKSVFKSKANGPGLVKCLSWLHYTNILMCNIYIPKHVSKSITGFGYLVPRSMSSQASKLLGVIFDSDIETAMTPNFTEANITAINSNSASPKQLQKFSDQFVNNDLPKYTKLTLMLGGHYLKSEADMPGSAESKHAVKAILSNHLNIDLDEFASLPDFKMEITKIPNCIPQYEVGYLDLKRKVQNAASKEFNDQISFGGMAFGDGVGIPDCVQNAFKDSATLSGI

SEQ ID NO: 8 - protein, 374 aa, synthetic construct
MLNRRFQSTVSSSLNKGTGIVFMNMGGPSTVKETYDFLFRLFSDGDLIPFGRFQNILARFIASRRTPKIESYYKAIGGGSPIRKWSEYQSSKLCEKLDIISPQSAPHKPYVAFRYANPLTEDTLQKMKNDGITKAIAFSQYPQFSYSTTGSSINELYRQSKILDPDQSIKWTVIDRWPDHPALVKTFAAHIKDTLNRFKTENGLTDTKDVVLQFSAHSLPMDIVNKGDSYPAEVAASVFAIMKELNFSNPYKLTWQSQVGPKPWLGAQTEKITKQLASSDVPGVVLVPIAFTSDHIETLHELDIELIQELPNPSKVKRVESLNGDQTFIDSLAELVKSHIDSKVVFSNQLPLDSMLGVVSDNSLTDPKEFFRAH

SEQ ID NO: 9 - protein, 145 aa, synthetic construct
MGAFTEKQEALVSSSFEAFKANIPQYSVVFYTSILEKAPAAKDLFSFLSNGVDPSNPKLTGHAEKLFGLVRDSAGQLKANGTVVADAALGSIHAQKAITDPQFVVVKEALLKTIKEAVGDKWSDELSSAWEVAYDELAAAIKKAF

SEQ ID NO: 10 - protein, 1155 aa, synthetic construct
MSNLPPTFGSTRQSPEDQSPPVPKELSFNGTTPSGKLRLFVCQTCTRAFARQEHLKRHERSHTKEKPFSCGICSRKFSRRDLLLRHAQKLHSNCSDAAITRLRRKATRRSSNAAGSISGSTPVTTPNTMGTPEDGEKRKVQKLAGRRDSNEQKLQLQQQHLQQQPQLQYQQSLKQHENQVQQPDQDPLISPRMQLFNDSNHHVNNLFDLGLRRASFSAVSGNNYAHYVNNFQQDASSTNPNQDSNNAEFENIEFSTPQMMPVEDAETWMNNMGPIPNFSLDVNRNIGDSFTDIQHKNSEPIISEPPKDTAPNDKKLNGYSFYEAPIKPLESLFSVRNTKRNKYKTNDDSPDTVDNNSAPAANTIQELESSLNASKNFCLPTGYSFYGNLDQQTFSNTLSCTSSNATISPILLDNSINNNSTSDVRPEFRTQSVTSEMSQAPPPPQKNNSKYSTEVLFTSNMRSFIHYALSKYPFIGVPTPTLPENERLNEYADSFTNRFLNHYPFIHVTILKEYSLFKAILDENESTKNWENNQFYLENQRISIVCLPLLVATIGAVLSNNKKDASNLYEASRRCIHVYLDSRKKIPTSLSANNNDSPLWLIQSLTLSVMYGLFADNDISLNVVIRQVNALNSLVKTSGLNRTSIIDLFNINKPLDNELWNQFVKIESTVRTIHTIFQISSNLSALYNIIPSLKIDDLMITLPVPTTLWQADSFVKFKSLSYGNQIPFQYTRVLQNLIDYNQPLSDGKFLYENHVSEFGLICLQNGLHQYSYFQKLTAVNNREDALFTKVVNSLHSWDRMISNSDLFPKKIYQQSCLILDSKLLNNFLIVKSSLKVSTGDVSSLNKLKENVWLKNWNQVCAIYYNSFMNIPAPSIQKKYNDIEFVDDMINLSLIIIKIMKLIFYNNVKDNYEDENDFKLQELNLTFDNFDEKISLNLTILFDIFLMIYKIITNYEKFMKIKHKFNYYNSNSNISFLHHFELSSVINNTQMNQNDYMKTDIDEKLDQLFHIYQTFFRLYLDLEKFMKFKFNYHDFETEFSSLSISNILNTHAASNNDTNAADAMNAKDEKISPTTLNSVLLADEGNENSGRNNDSDRLFMLNELINFEVGLKFLKIGESFFDFLYENNYKFIHFKNLNDGMFHIRIYLENRLDGGV

SEQ ID NO: 11 - protein, 888 aa, synthetic construct
MSTAAPIKEESQFAHLTLMNKDIPSNAKQAKSKVSAAPAKTGSKSAGGSGNNNAAPVKKRVRTGCLTCRKKHKKCDENRNPKCDFCTLKGLECVWPENNKKNIFVNNSMKDFLGKKTVDGADSLNLAVNLQQQQSSNTIANQSLSSIGLESFGYGSGIKNEFNFQDLIGSNSGSSDPTFSVDADEAQKLDISNKNSRKRQKLGLLPVSNATSHLNGFNGMSNGKSHSFSSPSGTNDDELSGLMFNSPSFNPLTVNDSTNNSNHNIGLSPMSCLFSTVQEASQKKHGNSSRHFSYPSGPEDLWFNEFQKQALTANGENAVQQGDDASKNNTAIPKDQSSNSSIFSSRSSAASSNSGDDIGRMGPFSKGPEIEFNYDSFLESLKAESPSSSKYNLPETLKEYMTLSSSHLNSQHSDTLANGTNGNYSSTVSNNLSLSLNSFSFSDKFSLSPPTITDAEKFSLMRNFIDNISPWFDTFDNTKQFGTKIPVLAKKCSSLYYAILAISSRQRERIKKEHNEKTLQCYQYSLQQLIPTVQSSNNIEYIITCILLSVFHIMSSEPSTQRDIIVSLAKYIQACNINGFTSNDKLEKSIFWNYVNLDLATCAIGEESMVIPFSYWVKETTDYKTIQDVKPFFTKKTSTTTDDDLDDMYAIYMLYISGRIINLLNCRDAKLNFEPKWEFLWNELNEWELNKPLTFQSIVQFKANDESQGGSTFPTVLFSNSRSCYSNQLYHMSYIILVQNKPRLYKIPFTTVSASMSSPSDNKAGMSASSTPASDHHASGDHLSPRSVEPSLSTTLSPPPNANGAGNKFRSTLWHAKQICGISINNNHNSNLAAKVNSLQPLWHAGKLISSKSEHTQLLKLLNNLECATGWPMNWKGKELIDYWNVEE

SEQ ID NO: 12 - protein, 989 aa, synthetic construct
MPPKHRLEQSIQPMASQQIVPGNKVILPNPKVDAKSTPNISVQKRRRVTRACDECRKKKVKCDGQQPCIHCTVYSYECTYSQPSSKKRQGQSLSLSAPSNINATSSVQKSVKPPEIDFQRMRDALKYYEDLLNQLIYPNSAPTVRVNPIRLASILKQLRADKSSDELISVKALSDNYIEMLHKTMQQPVQQPAPPSLGQGGSFSNHSPNHNNASIDGSIESNLGREIRIILPPRDIALKLIYKTWDNACVLFRFYHRPAFIEDLNELYETDLANYTNKQQRFLPLVYSVMACGALFCKTDGINHGQKSSKPKDSSDESLIDDEGYKYFIAARKLIDITDTRDTYGIQTIVMLIIFLQCSARLSTCYSYIGIALRAALREGLHRQLNYPFNPIELETRKRLFWTIYKMDIYVNTMLGLPRTISEEDFDQEMPIELDDENISETGYRFDLQGTKLSSSGIANAHTRLIFIMKKIVKKLYPVKLQKPTSNSGDTPLENNDLLAHEIVHELEMDLQNWVNSLPAELKPGIEPPTEYFKANRLLHLAYLHVKIILYRPFIHYISEKDKVGNSSIPPSPEEITSIEKAKNCVNVARIVVKLAEDMINRKMLSGSYWFSIYTIFFSVACLVYYVHFAPPKKDNGELDPQYMEIKKDTESGREVLNILKDSSMAARRTYNILNSLFEQLNRRTAKVNLAKAQQPPSGLNNPAATQYQKQGEHRQLQPSNYSGTVKSVDPENIDYSSFGSQFENTNIEDGSSNTKIDQKVNGVNYIDGVFTGINLNMPNLSETSNTQGIDNPAFQSINNSNLNNNFVQTKYIPGMMDQLDMKIFGRFLPPYMLNSNKVEQGQNERNLSGQPSSSNTPDGSQPVTVLDGLYPLQNDNNNNHDPGNSKSVVNNSNSVENLLQNFTMVPSGLSSTVQNPEAAQKFNNHMSNISNMNDPRRASVATSDGSNDMDHHSQGPINKDLKPLSNYEFDDLFFNDWTTAPDTINFDS

SEQ ID NO: 13 - protein, 684 aa, synthetic construct
MSISRDDDHPRPKRARSGKPKKETPPAKRRVRTGCLTCRRKHKKCDENRPKCDFCTAKGLECVWPEEVKKNVFVNNSFKDFCFSQSKHRDRFRKPTDFDLSSSLSPLDYHLGPDDPRTRKKAYSLDVADHYLSAFDGYSRKNEYLDAPLTTAYPLLETSESPLSGLFNAPQELPSQLTRTPSFGASSLSYFDTLQSYSMNPSLSSGSNDKISTASSVSSDMSLAKKDADFEHRYSFAEPQKKSKFGLDYYDLPNTLNDLMCLFIATKDSTSGSKLPNNETIFEIFTDKSTMEAPSIDDHEMMLLMETYIDQIAHFLNKSDETQCNIFMTKIPELAHRFPSLKYAILGLASRHLEKVRSDYSGEKTLQYYTYSLQQLSMCLNSDKNTLEVVATCVLLCYFEILSTNPDSWHSRLENCGSMLKVCHINARSETELEKALFWSFAALDIGCCAVGDRKTVVRPEDWFGTDAPSSPTETGTALQSMLYLSCQIFQLVSSNDDQSEFDSCWKSLWKQLGDWERARSSNMRGFCFKRDNSFPETLFSSSTALCANQLFHTCCILMLQTKPRLVKLHEPEKQERTPDTLFQSAIKTEQGESVSTSSLMSRSQIWHAKQIIGINVCNMKSASSRSLGCQILSLQAIWIAGKLISSAHEHSIILQLLQRLESWSSMSMDWREKQLTEFWKREC

SEQ ID NO: 14 - protein, 712 aa, synthetic construct
MSNLPPTFGSTRQSPEDQSPPVPKELSFNGTTPSGKLRLFVCQTCTRAFARQEHLKRHERSHTKEKPFSCGICSRKFSRRDLLLRHAQKLHSNCSDAAITRLRRKATRRSSNAAGSISGSTPVTTPNTMGTPEDGEKRKVQKLAGRRDSNEQKLQLQQQHLQQQPQLQYQQSLKQHENQVQQPDQDPLISPRMQLFNDSNHHVNNLFDLGLRRASFSAVSGNNYAHYVNNFQQDASSTNPNQDSNNAEFENIEFSTPQMMPVEDAETWMNNMGPIPNFSLDVNRNIGDSFTDIQHKNSEPIISEPPKDTAPNDKKLNGYSFYEAPIKPLESLFSVRNTKRNKYKTNDDSPDTVDNNSAPAANTIQELESSLNASKNFCLPTGYSFYGNLDQQTFSNTLSCGGGGSTSDAAITRLRRKATRRSSNAAGSISGSTPVTTPNTMGTPEDGEKRKVQKLAGRRDSNEQKLQLQQQHLQQQPQLQYQQSLKQHENQVQQPDQDPLISPRMQLFNDSNHHVNNLFDLGLRRASFSAVSGNNYAHYVNNFQQDASSTNPNQDSNNAEFENIEFSTPQMMPVEDAETWMNNMGPIPNFSLDVNRNIGDSFTDIQHKNSEPIISEPPKDTAPNDKKLNGYSFYEAPIKPLESLFSVRNTKRNKYKTNDDSPDTVDNNSAPAANTIQELESSLNASKNFCLPTGYSFYGNLDQQTFSNTLSC

SEQ ID NO: 15 - protein, 2060 aa, synthetic construct
MSNLPPTFGSTRQSPEDQSPPVPKELSFNGTTPSGKLRLFVCQTCTRAFARQEHLKRHERSHTKEKPFSCGICSRKFSRRDLLLRHAQKLHSNCSDAAITRLRRKATRRSSNAAGSISGSTPVTTPNTMGTPEDGEKRKVQKLAGRRDSNEQKLQLQQQHLQQQPQLQYQQSLKQHENQVQQPDQDPLISPRMQLFNDSNHHVNNLFDLGLRRASFSAVSGNNYAHYVNNFQQDASSTNPNQDSNNAEFENIEFSTPQMMPVEDAETWMNNMGPIPNFSLDVNRNIGDSFTDIQHKNSEPIISEPPKDTAPNDKKLNGYSFYEAPIKPLESLFSVRNTKRNKYKTNDDSPDTVDNNSAPAANTIQELESSLNASKNFCLPTGYSFYGNLDQQTFSNTLSCTSSNATISPILLDNSINNNSTSDVRPEFRTQSVTSEMSQAPPPPQKNNSKYSTEVLFTSNMRSFIHYALSKYPFIGVPTPTLPENERLNEYADSFTNRFLNHYPFIHVTILKEYSLFKAILDENESTKNWENNQFYLENQRISIVCLPLLVATIGAVLSNNKKDASNLYEASRRCIHVYLDSRKKIPTSLSANNNDSPLWLIQSLTLSVMYGLFADNDISLNVVIRQVNALNSLVKTSGLNRTSIIDLFNINKPLDNELWNQFVKIESTVRTIHTIFQISSNLSALYNIIPSLKIDDLMITLPVPTTLWQADSFVKFKSLSYGNQIPFQYTRVLQNLIDYNQPLSDGKFLYENHVSEFGLICLQNGLHQYSYFQKLTAVNNREDALFTKVVNSLHSWDRMISNSDLFPKKIYQQSCLILDSKLLNNFLIVKSSLKVSTGDVSSLNKLKENVWLKNWNQVCAIYYNSFMNIPAPSIQKKYNDIEFVDDMINLSLIIIKIMKLIFYNNVKDNYEDENDFKLQELNLTFDNFDEKISLNLTILFDIFLMIYKIITNYEKFMKIKHKFNYYNSNSNISFLHHFELSSVINNTQMNQNDYMKTDIDEKLDQLFHIYQTFFRLYLDLEKFMKFKFNYHDFETEFSSLSISNILNTHAASNNDTNAADAMNAKDEKISPTTLNSVLLADEGNENSGRNNDSDRLFMLNELINFEVGLKFLKIGESFFDFLYENNYKFIHFKNLNDGMFHIRIYLENRLDGGVGGGGSGQSLSLSAPSNINATSSVQKSVKPPEIDFQRMRDALKYYEDLLNQLIYPNSAPTVRVNPIRLASILKQLRADKSSDELISVKALSDNYIEMLHKTMQQPVQQPAPPSLGQGGSFSNHSPNHNNASIDGSIESNLGREIRIILPPRDIALKLIYKTWDNACVLFRFYHRPAFIEDLNELYETDLANYTNKQQRFLPLVYSVMACGALFCKTDGINHGQKSSKPKDSSDESLIDDEGYKYFIAARKLIDITDTRDTYGIQTIVMLIIFLQCSARLSTCYSYIGIALRAALREGLHRQLNYPFNPIELETRKRLFWTIYKMDIYVNTMLGLPRTISEEDFDQEMPIELDDENISETGYRFDLQGTKLSSSGIANAHTRLIFIMKKIVKKLYPVKLQKPTSNSGDTPLENNDLLAHEIVHELEMDLQNWVNSLPAELKPGIEPPTEYFKANRLLHLAYLHVKIILYRPFIHYISEKDKVGNSSIPPSPEEITSIEKAKNCVNVARIVVKLAEDMINRKMLSGSYWFSIYTIFFSVACLVYYVHFAPPKKDNGELDPQYMEIKKDTESGREVLNILKDSSMAARRTYNILNSLFEQLNRRTAKVNLAKAQQPPSGLNNPAATQYQKQGEHRQLQPSNYSGTVKSVDPENIDYSSFGSQFENTNIEDGSSNTKIDQKVNGVNYIDGVFTGINLNMPNLSETSNTQGIDNPAFQSINNSNLNNNFVQTKYIPGMMDQLDMKIFGRFLPPYMLNSNKVEQGQNERNLSGQPSSSNTPDGSQPVTVLDGLYPLQNDNNNNHDPGNSKSVVNNSNSVENLLQNFTMVPSGLSSTVQNPEAAQKFNNHMSNISNMNDPRRASVATSDGSNDMDHHSQGPINKDLKPLSNYEFDDLFFNDWTTAPDTINFDS

SEQ ID NO: 16 - protein, 884 aa, synthetic construct
MSNLPPTFGSTRQSPEDQSPPVPKELSFNGTTPSGKLRLFVCQTCTRAFARQEHLKRHERSHTKEKPFSCGICSRKFSRRDLLLRHAQKLHSNCSGGGGSVNNSMKDFLGKKTVDGADSLNLAVNLQQQQSSNTIANQSLSSIGLESFGYGSGIKNEFNFQDLIGSNSGSSDPTFSVDADEAQKLDISNKNSRKRQKLGLLPVSNATSHLNGFNGMSNGKSHSFSSPSGTNDDELSGLMFNSPSFNPLTVNDSTNNSNHNIGLSPMSCLFSTVQEASQKKHGNSSRHFSYPSGPEDLWFNEFQKQALTANGENAVQQGDDASKNNTAIPKDQSSNSSIFSSRSSAASSNSGDDIGRMGPFSKGPEIEFNYDSFLESLKAESPSSSKYNLPETLKEYMTLSSSHLNSQHSDTLANGTNGNYSSTVSNNLSLSLNSFSFSDKFSLSPPTITDAEKFSLMRNFIDNISPWFDTFDNTKQFGTKIPVLAKKCSSLYYAILAISSRQRERIKKEHNEKTLQCYQYSLQQLIPTVQSSNNIEYIITCILLSVFHIMSSEPSTQRDIIVSLAKYIQACNINGFTSNDKLEKSIFWNYVNLDLATCAIGEESMVIPFSYWVKETTDYKTIQDVKPFFTKKTSTTTDDDLDDMYAIYMLYISGRIINLLNCRDAKLNFEPKWEFLWNELNEWELNKPLTFQSIVQFKANDESQGGSTFPTVLFSNSRSCYSNQLYHMSYIILVQNKPRLYKIPFTTVSASMSSPSDNKAGMSASSTPASDHHASGDHLSPRSVEPSLSTTLSPPPNANGAGNKFRSTLWHAKQICGISINNNHNSNLAAKVNSLQPLWHAGKLISSKSEHTQLLKLLNNLECATGWPMNWKGKELIDYWNVEE

SEQ ID NO: 17 - protein, 1000 aa, synthetic construct
MSNLPPTFGSTRQSPEDQSPPVPKELSFNGTTPSGKLRLFVCQTCTRAFARQEHLKRHERSHTKEKPFSCGICSRKFSRRDLLLRHAQKLHSNCSGGGGSGQSLSLSAPSNINATSSVQKSVKPPEIDFQRMRDALKYYEDLLNQLIYPNSAPTVRVNPIRLASILKQLRADKSSDELISVKALSDNYIEMLHKTMQQPVQQPAPPSLGQGGSFSNHSPNHNNASIDGSIESNLGREIRIILPPRDIALKLIYKTWDNACVLFRFYHRPAFIEDLNELYETDLANYTNKQQRFLPLVYSVMACGALFCKTDGINHGQKSSKPKDSSDESLIDDEGYKYFIAARKLIDITDTRDTYGIQTIVMLIIFLQCSARLSTCYSYIGIALRAALREGLHRQLNYPFNPIELETRKRLFWTIYKMDIYVNTMLGLPRTISEEDFDQEMPIELDDENISETGYRFDLQGTKLSSSGIANAHTRLIFIMKKIVKKLYPVKLQKPTSNSGDTPLENNDLLAHEIVHELEMDLQNWVNSLPAELKPGIEPPTEYFKANRLLHLAYLHVKIILYRPFIHYISEKDKVGNSSIPPSPEEITSIEKAKNCVNVARIVVKLAEDMINRKMLSGSYWFSIYTIFFSVACLVYYVHFAPPKKDNGELDPQYMEIKKDTESGREVLNILKDSSMAARRTYNILNSLFEQLNRRTAKVNLAKAQQPPSGLNNPAATQYQKQGEHRQLQPSNYSGTVKSVDPENIDYSSFGSQFENTNIEDGSSNTKIDQKVNGVNYIDGVFTGINLNMPNLSETSNTQGIDNPAFQSINNSNLNNNFVQTKYIPGMMDQLDMKIFGRFLPPYMLNSNKVEQGQNERNLSGQPSSSNTPDGSQPVTVLDGLYPLQNDNNNNHDPGNSKSVVNNSNSVENLLQNFTMVPSGLSSTVQNPEAAQKFNNHMSNISNMNDPRRASVATSDGSNDMDHHSQGPINKDLKPLSNYEFDDLFFNDWTTAPDTINFDS

SEQ ID NO: 18 - protein, 1198 aa, synthetic construct
MSTAAPIKEESQFAHLTLMNKDIPSNAKQAKSKVSAAPAKTGSKSAGGSGNNNAAPVKKRVRTGCLTCRKKHKKCDENRNPKCDFCTLKGLECVWPENNKKNIFVNNSMKDFLGKKTVDGADSLNLAVNLQQQQSSNTIANQSLSSIGLESFGYGSGIKNEFNFQDLIGSNSGSSDPTFSVDADEAQKLDISNKNSRKRQKLGLLPVSNATSHLNGFNGMSNGKSHSFSSPSGTNDDELSGLMFNSPSFNPLTVNDSTNNSNHNIGLSPMSCLFSTVQEASQKKHGNSSRHFSYPSGPEDLWFNEFQKQALTANGENAVQQGDDASKNNTAIPKDQSSNSSIFSSRSSAASSNSGDDIGRMGPFSKGPEIEFNYDSFLESLKAESPSSSKYNLPETLKEYMTLSSSHLNSQHSDTLANGTNGNYSSTVSNNLSLSLNSFSFSDKFSLSPPTITDAEKFSLMRNFIDNISPWFDTFDNTKQFGTKIPVLAKKCSSLYYAILAISSRQRERIKKEHNEKTLQCYQYSLQQLIPTVQSSNNIEYIITCILLSVFHIMSSEPSTQRDIIVSLAKYIQACNINGFTSNDKLEKSIFWNYVNLDLATCAIGEESMVIPFSYWVKETTDYKTIQDVKPFFTKKTSTTTDDDLDDMYAIYMLYISGRIINLLNCRDAKLNFEPKWEFLWNELNEWELNKPLTFQSIVQFKANDESQGGSTFPTVLFSNSRSCYSNQLYHMSYIILVQNKPRLYKIPFTTVSASMSSPSDNKAGMSASSTPASDHHASGDHLSPRSVEPSLSTTLSPPPNANGAGNKFRSTLWHAKQICGISINNNHNSNLAAKVNSLQPLWHAGKLISSKSEHTQLLKLLNNLECATGWPMNWKGKELIDYWNVEEGGGGSDAAITRLRRKATRRSSNAAGSISGSTPVTTPNTMGTPEDGEKRKVQKLAGRRDSNEQKLQLQQQHLQQQPQLQYQQSLKQHENQVQQPDQDPLISPRMQLFNDSNHHVNNLFDLGLRRASFSAVSGNNYAHYVNNFQQDASSTNPNQDSNNAEFENIEFSTPQMMPVEDAETWMNNMGPIPNFSLDVNRNIGDSFTDIQHKNSEPIISEPPKDTAPNDKKLNGYSFYEAPIKPLESLFSVRNTKRNKYKTNDDSPDTVDNNSAPAANTIQELESSLNASKNFCLPTGYSFYGNLDQQTFSNTLSC

SEQ ID NO: 19 - protein, 418 aa, synthetic construct
MSTAAPIKEESQFAHLTLMNKDIPSNAKQAKSKVSAAPAKTGSKSAGGSGNNNAAPVKKRVRTGCLTCRKKHKKCDENRNPKCDFCTLKGLECVWPENNKKNIFGGGGSSNCSDAAITRLRRKATRRSSNAAGSISGSTPVTTPNTMGTPEDGEKRKVQKLAGRRDSNEQKLQLQQQHLQQQPQLQYQQSLKQHENQVQQPDQDPLISPRMQLFNDSNHHVNNLFDLGLRRASFSAVSGNNYAHYVNNFQQDASSTNPNQDSNNAEFENIEFSTPQMMPVEDAETWMNNMGPIPNFSLDVNRNIGDSFTDIQHKNSEPIISEPPKDTAPNDKKLNGYSFYEAPIKPLESLFSVRNTKRNKYKTNDDSPDTVDNNSAPAANTIQELESSLNASKNFCLPTGYSFYGNLDQQTFSNTLSC

SEQ ID NO: 20 - protein, 1173 aa, synthetic construct
MSTAAPIKEESQFAHLTLMNKDIPSNAKQAKSKVSAAPAKTGSKSAGGSGNNNAAPVKKRVRTGCLTCRKKHKKCDENRNPKCDFCTLKGLECVWPENNKKNIFGGGGSSNCSDAAITRLRRKATRRSSNAAGSISGSTPVTTPNTMGTPEDGEKRKVQKLAGRRDSNEQKLQLQQQHLQQQPQLQYQQSLKQHENQVQQPDQDPLISPRMQLFNDSNHHVNNLFDLGLRRASFSAVSGNNYAHYVNNFQQDASSTNPNQDSNNAEFENIEFSTPQMMPVEDAETWMNNMGPIPNFSLDVNRNIGDSFTDIQHKNSEPIISEPPKDTAPNDKKLNGYSFYEAPIKPLESLFSVRNTKRNKYKTNDDSPDTVDNNSAPAANTIQELESSLNASKNFCLPTGYSFYGNLDQQTFSNTLSCTSSNATISPILLDNSINNNSTSDVRPEFRTQSVTSEMSQAPPPPQKNNSKYSTEVLFTSNMRSFIHYALSKYPFIGVPTPTLPENERLNEYADSFTNRFLNHYPFIHVTILKEYSLFKAILDENESTKNWENNQFYLENQRISIVCLPLLVATIGAVLSNNKKDASNLYEASRRCIHVYLDSRKKIPTSLSANNNDSPLWLIQSLTLSVMYGLFADNDISLNVVIRQVNALNSLVKTSGLNRTSIIDLFNINKPLDNELWNQFVKIESTVRTIHTIFQISSNLSALYNIIPSLKIDDLMITLPVPTTLWQADSFVKFKSLSYGNQIPFQYTRVLQNLIDYNQPLSDGKFLYENHVSEFGLICLQNGLHQYSYFQKLTAVNNREDALFTKVVNSLHSWDRMISNSDLFPKKIYQQSCLILDSKLLNNFLIVKSSLKVSTGDVSSLNKLKENVWLKNWNQVCAIYYNSFMNIPAPSIQKKYNDIEFVDDMINLSLIIIKIMKLIFYNNVKDNYEDENDFKLQELNLTFDNFDEKISLNLTILFDIFLMIYKIITNYEKFMKIKHKFNYYNSNSNISFLHHFELSSVINNTQMNQNDYMKTDIDEKLDQLFHIYQTFFRLYLDLEKFMKFKFNYHDFETEFSSLSISNILNTHAASNNDTNAADAMNAKDEKISPTTLNSVLLADEGNENSGRNNDSDRLFMLNELINFEVGLKFLKIGESFFDFLYENNYKFIHFKNLNDGMFHIRIYLENRLDGGV

SEQ ID NO: 21 - protein, 1009 aa, synthetic construct
MSTAAPIKEESQFAHLTLMNKDIPSNAKQAKSKVSAAPAKTGSKSAGGSGNNNAAPVKKRVRTGCLTCRKKHKKCDENRNPKCDFCTLKGLECVWPENNKKNIFGGGGSGQSLSLSAPSNINATSSVQKSVKPPEIDFQRMRDALKYYEDLLNQLIYPNSAPTVRVNPIRLASILKQLRADKSSDELISVKALSDNYIEMLHKTMQQPVQQPAPPSLGQGGSFSNHSPNHNNASIDGSIESNLGREIRIILPPRDIALKLIYKTWDNACVLFRFYHRPAFIEDLNELYETDLANYTNKQQRFLPLVYSVMACGALFCKTDGINHGQKSSKPKDSSDESLIDDEGYKYFIAARKLIDITDTRDTYGIQTIVMLIIFLQCSARLSTCYSYIGIALRAALREGLHRQLNYPFNPIELETRKRLFWTIYKMDIYVNTMLGLPRTISEEDFDQEMPIELDDENISETGYRFDLQGTKLSSSGIANAHTRLIFIMKKIVKKLYPVKLQKPTSNSGDTPLENNDLLAHEIVHELEMDLQNWVNSLPAELKPGIEPPTEYFKANRLLHLAYLHVKIILYRPFIHYISEKDKVGNSSIPPSPEEITSIEKAKNCVNVARIVVKLAEDMINRKMLSGSYWFSIYTIFFSVACLVYYVHFAPPKKDNGELDPQYMEIKKDTESGREVLNILKDSSMAARRTYNILNSLFEQLNRRTAKVNLAKAQQPPSGLNNPAATQYQKQGEHRQLQPSNYSGTVKSVDPENIDYSSFGSQFENTNIEDGSSNTKIDQKVNGVNYIDGVFTGINLNMPNLSETSNTQGIDNPAFQSINNSNLNNNFVQTKYIPGMMDQLDMKIFGRFLPPYMLNSNKVEQGQNERNLSGQPSSSNTPDGSQPVTVLDGLYPLQNDNNNNHDPGNSKSVVNNSNSVENLLQNFTMVPSGLSSTVQNPEAAQKFNNHMSNISNMNDPRRASVATSDGSNDMDHHSQGPINKDLKPLSNYEFDDLFFNDWTTAPDTINFDS

SEQ ID NO: 22 - protein, 1299 aa, synthetic construct
MPPKHRLEQSIQPMASQQIVPGNKVILPNPKVDAKSTPNISVQKRRRVTRACDECRKKKVKCDGQQPCIHCTVYSYECTYSQPSSKKRQGQSLSLSAPSNINATSSVQKSVKPPEIDFQRMRDALKYYEDLLNQLIYPNSAPTVRVNPIRLASILKQLRADKSSDELISVKALSDNYIEMLHKTMQQPVQQPAPPSLGQGGSFSNHSPNHNNASIDGSIESNLGREIRIILPPRDIALKLIYKTWDNACVLFRFYHRPAFIEDLNELYETDLANYTNKQQRFLPLVYSVMACGALFCKTDGINHGQKSSKPKDSSDESLIDDEGYKYFIAARKLIDITDTRDTYGIQTIVMLIIFLQCSARLSTCYSYIGIALRAALREGLHRQLNYPFNPIELETRKRLFWTIYKMDIYVNTMLGLPRTISEEDFDQEMPIELDDENISETGYRFDLQGTKLSSSGIANAHTRLIFIMKKIVKKLYPVKLQKPTSNSGDTPLENNDLLAHEIVHELEMDLQNWVNSLPAELKPGIEPPTEYFKANRLLHLAYLHVKIILYRPFIHYISEKDKVGNSSIPPSPEEITSIEKAKNCVNVARIVVKLAEDMINRKMLSGSYWFSIYTIFFSVACLVYYVHFAPPKKDNGELDPQYMEIKKDTESGREVLNILKDSSMAARRTYNILNSLFEQLNRRTAKVNLAKAQQPPSGLNNPAATQYQKQGEHRQLQPSNYSGTVKSVDPENIDYSSFGSQFENTNIEDGSSNTKIDQKVNGVNYIDGVFTGINLNMPNLSETSNTQGIDNPAFQSINNSNLNNNFVQTKYIPGMMDQLDMKIFGRFLPPYMLNSNKVEQGQNERNLSGQPSSSNTPDGSQPVTVLDGLYPLQNDNNNNHDPGNSKSVVNNSNSVENLLQNFTMVPSGLSSTVQNPEAAQKFNNHMSNISNMNDPRRASVATSDGSNDMDHHSQGPINKDLKPLSNYEFDDLFFNDWTTAPDTINFDSGGGGSDAAITRLRRKATRRSSNAAGSISGSTPVTTPNTMGTPEDGEKRKVQKLAGRRDSNEQKLQLQQQHLQQQPQLQYQQSLKQHENQVQQPDQDPLISPRMQLFNDSNHHVNNLFDLGLRRASFSAVSGNNYAHYVNNFQQDASSTNPNQDSNNAEFENIEFSTPQMMPVEDAETWMNNMGPIPNFSLDVNRNIGDSFTDIQHKNSEPIISEPPKDTAPNDKKLNGYSFYEAPIKPLESLFSVRNTKRNKYKTNDDSPDTVDNNSAPAANTIQELESSLNASKNFCLPTGYSFYGNLDQQTFSNTLSC

SEQ ID NO: 23 - protein, 403 aa, synthetic construct
MPPKHRLEQSIQPMASQQIVPGNKVILPNPKVDAKSTPNISVQKRRRVTRACDECRKKKVKCDGQQPCIHCTVYSYECTYSQPSSKKRQGGGGSSNCSDAAITRLRRKATRRSSNAAGSISGSTPVTTPNTMGTPEDGEKRKVQKLAGRRDSNEQKLQLQQQHLQQQPQLQYQQSLKQHENQVQQPDQDPLISPRMQLFNDSNHHVNNLFDLGLRRASFSAVSGNNYAHYVNNFQQDASSTNPNQDSNNAEFENIEFSTPQMMPVEDAETWMNNMGPIPNFSLDVNRNIGDSFTDIQHKNSEPIISEPPKDTAPNDKKLNGYSFYEAPIKPLESLFSVRNTKRNKYKTNDDSPDTVDNNSAPAANTIQELESSLNASKNFCLPTGYSFYGNLDQQTFSNTLSC

SEQ ID NO: 24 - protein, 1158 aa, synthetic construct
MPPKHRLEQSIQPMASQQIVPGNKVILPNPKVDAKSTPNISVQKRRRVTRACDECRKKKVKCDGQQPCIHCTVYSYECTYSQPSSKKRQGGGGSSNCSDAAITRLRRKATRRSSNAAGSISGSTPVTTPNTMGTPEDGEKRKVQKLAGRRDSNEQKLQLQQQHLQQQPQLQYQQSLKQHENQVQQPDQDPLISPRMQLFNDSNHHVNNLFDLGLRRASFSAVSGNNYAHYVNNFQQDASSTNPNQDSNNAEFENIEFSTPQMMPVEDAETWMNNMGPIPNFSLDVNRNIGDSFTDIQHKNSEPIISEPPKDTAPNDKKLNGYSFYEAPIKPLESLFSVRNTKRNKYKTNDDSPDTVDNNSAPAANTIQELESSLNASKNFCLPTGYSFYGNLDQQTFSNTLSCTSSNATISPILLDNSINNNSTSDVRPEFRTQSVTSEMSQAPPPPQKNNSKYSTEVLFTSNMRSFIHYALSKYPFIGVPTPTLPENERLNEYADSFTNRFLNHYPFIHVTILKEYSLFKAILDENESTKNWENNQFYLENQRISIVCLPLLVATIGAVLSNNKKDASNLYEASRRCIHVYLDSRKKIPTSLSANNNDSPLWLIQSLTLSVMYGLFADNDISLNVVIRQVNALNSLVKTSGLNRTSIIDLFNINKPLDNELWNQFVKIESTVRTIHTIFQISSNLSALYNIIPSLKIDDLMITLPVPTTLWQADSFVKFKSLSYGNQIPFQYTRVLQNLIDYNQPLSDGKFLYENHVSEFGLICLQNGLHQYSYFQKLTAVNNREDALFTKVVNSLHSWDRMISNSDLFPKKIYQQSCLILDSKLLNNFLIVKSSLKVSTGDVSSLNKLKENVWLKNWNQVCAIYYNSFMNIPAPSIQKKYNDIEFVDDMINLSLIIIKIMKLIFYNNVKDNYEDENDFKLQELNLTFDNFDEKISLNLTILFDIFLMIYKIITNYEKFMKIKHKFNYYNSNSNISFLHHFELSSVINNTQMNQNDYMKTDIDEKLDQLFHIYQTFFRLYLDLEKFMKFKFNYHDFETEFSSLSISNILNTHAASNNDTNAADAMNAKDEKISPTTLNSVLLADEGNENSGRNNDSDRLFMLNELINFEVGLKFLKIGESFFDFLYENNYKFIHFKNLNDGMFHIRIYLENRLDGGV

SEQ ID NO: 25 - protein, 878 aa, synthetic construct
MPPKHRLEQSIQPMASQQIVPGNKVILPNPKVDAKSTPNISVQKRRRVTRACDECRKKKVKCDGQQPCIHCTVYSYECTYSQPSSKKRQGGGGSVNNSMKDFLGKKTVDGADSLNLAVNLQQQQSSNTIANQSLSSIGLESFGYGSGIKNEFNFQDLIGSNSGSSDPTFSVDADEAQKLDISNKNSRKRQKLGLLPVSNATSHLNGFNGMSNGKSHSFSSPSGTNDDELSGLMFNSPSFNPLTVNDSTNNSNHNIGLSPMSCLFSTVQEASQKKHGNSSRHFSYPSGPEDLWFNEFQKQALTANGENAVQQGDDASKNNTAIPKDQSSNSSIFSSRSSAASSNSGDDIGRMGPFSKGPEIEFNYDSFLESLKAESPSSSKYNLPETLKEYMTLSSSHLNSQHSDTLANGTNGNYSSTVSNNLSLSLNSFSFSDKFSLSPPTITDAEKFSLMRNFIDNISPWFDTFDNTKQFGTKIPVLAKKCSSLYYAILAISSRQRERIKKEHNEKTLQCYQYSLQQLIPTVQSSNNIEYIITCILLSVFHIMSSEPSTQRDIIVSLAKYIQACNINGFTSNDKLEKSIFWNYVNLDLATCAIGEESMVIPFSYWVKETTDYKTIQDVKPFFTKKTSTTTDDDLDDMYAIYMLYISGRIINLLNCRDAKLNFEPKWEFLWNELNEWELNKPLTFQSIVQFKANDESQGGSTFPTVLFSNSRSCYSNQLYHMSYIILVQNKPRLYKIPFTTVSASMSSPSDNKAGMSASSTPASDHHASGDHLSPRSVEPSLSTTLSPPPNANGAGNKFRSTLWHAKQICGISINNNHNSNLAAKVNSLQPLWHAGKLISSKSEHTQLLKLLNNLECATGWPMNWKGKELIDYWNVEE

SEQ ID NO: 26 - protein, 154 aa, synthetic construct
MGLSDGEWQLVLNAWGKVEADVAGHGQEVLIRLFTGHPETLEKFDKFKHLKTEAEMKASEDLKKHGNTVLTALGGILKKKGHHEAEVKHLAESHANKHKIPVKYLEFISDAIIHVLHAKHPSDFGADAQAAMSKALELFRNDMAAQYKVLGFHG

SEQ ID NO: 27 - protein, 5 aa, synthetic construct
  VARIANT 1..5: note = Can be present in repeats of any integer
GGGGS

SEQ ID NO: 28 - protein, 12 aa, synthetic construct
GSAGSAAGSGEF

SEQ ID NO: 29 - protein, 18 aa, synthetic construct
KESGSVSSEQLAQFRSLD

SEQ ID NO: 30 - protein, 14 aa, synthetic construct
EGKSSGSGSESKST

SEQ ID NO: 31 - protein, 5 aa, synthetic construct
  VARIANT 1..5: note = Can be present in repeats of any integer
EAAAK